European Patent Application EP 4 180 454 A1, published May 17, 2023. Title: 一种抗IgE的工程化抗体及其应用. Applicant: 上海济煜医药科技有限公司；江西济民可信集团有限公司. The sequence listing filed with the application follows.

SEQUENCE LISTING (64 sequences)

SEQ ID NO: 1 - protein, 23 aa, 人工序列（Artificial Sequence）
  LFR1
DIQLTQSPSSLSASVGDRVTITC

SEQ ID NO: 2 - protein, 15 aa, 人工序列（Artificial Sequence）
  LCDR1
RASQSVDYDGDSYMN

SEQ ID NO: 3 - protein, 15 aa, 人工序列（Artificial Sequence）
  LCDR1
RASQSVDYEGDSYMN

SEQ ID NO: 4 - protein, 15 aa, 人工序列（Artificial Sequence）
  LCDR1
RASQSLYDEGDSYMN

SEQ ID NO: 5 - protein, 15 aa, 人工序列（Artificial Sequence）
  LCDR1
RASQSVADEWDSYMN

SEQ ID NO: 6 - protein, 15 aa, 人工序列（Artificial Sequence）
  LCDR1
RASQSVDAEGDSYMN

SEQ ID NO: 7 - protein, 15 aa, 人工序列（Artificial Sequence）
  LCDR1
RASQSVDDEGDSYMN

SEQ ID NO: 8 - protein, 15 aa, 人工序列（Artificial Sequence）
  LCDR1
RASQSVDDEYDSYMN

SEQ ID NO: 9 - protein, 15 aa, 人工序列（Artificial Sequence）
  LCDR1
RASQSVDSEGDSYMN

SEQ ID NO: 10 - protein, 15 aa, 人工序列（Artificial Sequence）
  LCDR1
RASQSVEDEWDSYMN

SEQ ID NO: 11 - protein, 15 aa, 人工序列（Artificial Sequence）
  LCDR1
RASQSVFDEGDSYMN

SEQ ID NO: 12 - protein, 15 aa, 人工序列（Artificial Sequence）
  LCDR1
RASQSVGDEADSYMN

SEQ ID NO: 13 - protein, 15 aa, 人工序列（Artificial Sequence）
  LCDR1
RASQSVNDEADSYMN

SEQ ID NO: 14 - protein, 15 aa, 人工序列（Artificial Sequence）
  LCDR1
RASQSVNDEWDSYMN

SEQ ID NO: 15 - protein, 15 aa, 人工序列（Artificial Sequence）
  LFR2
WYQQKPGKAPKLLIY

SEQ ID NO: 16 - protein, 7 aa, 人工序列（Artificial Sequence）
  LCDR2
AASYLES

SEQ ID NO: 17 - protein, 7 aa, 人工序列（Artificial Sequence）
  LCDR2
AASYLQS

SEQ ID NO: 18 - protein, 32 aa, 人工序列（Artificial Sequence）
  LFR3
GVPSRFSGSGSGTDFTLTISSLQPEDFATYYC

SEQ ID NO: 19 - protein, 9 aa, 人工序列（Artificial Sequence）
  LCDR3
QQSHEDPYT

SEQ ID NO: 20 - protein, 10 aa, 人工序列（Artificial Sequence）
  LFR4
FGQGTKVEIK

SEQ ID NO: 21 - protein, 10 aa, 人工序列（Artificial Sequence）
  LFR4
FGQGTKLEIK

SEQ ID NO: 22 - protein, 111 aa, 人工序列（Artificial Sequence） [sequence omitted]

SEQ ID NO: 23 - protein, 111 aa, 人工序列（Artificial Sequence）
  VL
DIQLTQSPSSLSASVGDRVTITCRASQSVDYEGDSYMNWYQQKPGKAPKLLIYAASYLQSGVPSRFSGSGSGTDFTLTISSLQPEDFATYYCQQSHEDPYTFGQGTKLEIK

SEQ ID NO: 24 - protein, 111 aa, 人工序列（Artificial Sequence）
  VL
DIQLTQSPSSLSASVGDRVTITCRASQSLYDEGDSYMNWYQQKPGKAPKLLIYAASYLQSGVPSRFSGSGSGTDFTLTISSLQPEDFATYYCQQSHEDPYTFGQGTKLEIK

SEQ ID NO: 25 - protein, 111 aa, 人工序列（Artificial Sequence）
  VL
DIQLTQSPSSLSASVGDRVTITCRASQSVADEWDSYMNWYQQKPGKAPKLLIYAASYLQSGVPSRFSGSGSGTDFTLTISSLQPEDFATYYCQQSHEDPYTFGQGTKLEIK

SEQ ID NO: 26 - protein, 111 aa, 人工序列（Artificial Sequence）
  VL
DIQLTQSPSSLSASVGDRVTITCRASQSVDAEGDSYMNWYQQKPGKAPKLLIYAASYLQSGVPSRFSGSGSGTDFTLTISSLQPEDFATYYCQQSHEDPYTFGQGTKLEIK

SEQ ID NO: 27 - protein, 111 aa, 人工序列（Artificial Sequence）
  VL
DIQLTQSPSSLSASVGDRVTITCRASQSVDDEGDSYMNWYQQKPGKAPKLLIYAASYLQSGVPSRFSGSGSGTDFTLTISSLQPEDFATYYCQQSHEDPYTFGQGTKLEIK

SEQ ID NO: 28 - protein, 111 aa, 人工序列（Artificial Sequence）
  VL
DIQLTQSPSSLSASVGDRVTITCRASQSVDDEYDSYMNWYQQKPGKAPKLLIYAASYLQSGVPSRFSGSGSGTDFTLTISSLQPEDFATYYCQQSHEDPYTFGQGTKLEIK

SEQ ID NO: 29 - protein, 111 aa, 人工序列（Artificial Sequence）
  VL
DIQLTQSPSSLSASVGDRVTITCRASQSVDSEGDSYMNWYQQKPGKAPKLLIYAASYLQSGVPSRFSGSGSGTDFTLTISSLQPEDFATYYCQQSHEDPYTFGQGTKLEIK

SEQ ID NO: 30 - protein, 111 aa, 人工序列（Artificial Sequence）
  VL
DIQLTQSPSSLSASVGDRVTITCRASQSVEDEWDSYMNWYQQKPGKAPKLLIYAASYLQSGVPSRFSGSGSGTDFTLTISSLQPEDFATYYCQQSHEDPYTFGQGTKLEIK

SEQ ID NO: 31 - protein, 111 aa, 人工序列（Artificial Sequence）
  VL
DIQLTQSPSSLSASVGDRVTITCRASQSVFDEGDSYMNWYQQKPGKAPKLLIYAASYLQSGVPSRFSGSGSGTDFTLTISSLQPEDFATYYCQQSHEDPYTFGQGTKLEIK

SEQ ID NO: 32 - protein, 111 aa, 人工序列（Artificial Sequence）
  VL
DIQLTQSPSSLSASVGDRVTITCRASQSVGDEADSYMNWYQQKPGKAPKLLIYAASYLQSGVPSRFSGSGSGTDFTLTISSLQPEDFATYYCQQSHEDPYTFGQGTKLEIK

SEQ ID NO: 33 - protein, 111 aa, 人工序列（Artificial Sequence）
  VL
DIQLTQSPSSLSASVGDRVTITCRASQSVNDEADSYMNWYQQKPGKAPKLLIYAASYLQSGVPSRFSGSGSGTDFTLTISSLQPEDFATYYCQQSHEDPYTFGQGTKLEIK

SEQ ID NO: 34 - protein, 111 aa, 人工序列（Artificial Sequence）
  VL
DIQLTQSPSSLSASVGDRVTITCRASQSVNDEWDSYMNWYQQKPGKAPKLLIYAASYLQSGVPSRFSGSGSGTDFTLTISSLQPEDFATYYCQQSHEDPYTFGQGTKLEIK

SEQ ID NO: 35 - protein, 25 aa, 人工序列（Artificial Sequence） [sequence omitted]

SEQ ID NO: 36 - protein, 8 aa, 人工序列（Artificial Sequence）
  HCDR1
GYSITSGY

SEQ ID NO: 37 - protein, 8 aa, 人工序列（Artificial Sequence）
  HCDR1
GYSIRSGY

SEQ ID NO: 38 - protein, 8 aa, 人工序列（Artificial Sequence）
  HCDR1
GYSITQGY

SEQ ID NO: 39 - protein, 19 aa, 人工序列（Artificial Sequence）
  HFR2
SWNWIRQAPGKGLEWVASI

SEQ ID NO: 40 - protein, 19 aa, 人工序列（Artificial Sequence）
  HFR2
SWNWVRQAPGKGLEWVSVI

SEQ ID NO: 41 - protein, 5 aa, 人工序列（Artificial Sequence）
  HCDR2
TYDGS

SEQ ID NO: 42 - protein, 5 aa, 人工序列（Artificial Sequence）
  HCDR2
TYAGS

SEQ ID NO: 43 - protein, 41 aa, 人工序列（Artificial Sequence）
  HFR3
TNYNPSVKGRITISRDDSKNTFYLQMNSLRAEDTAVYYCAR

SEQ ID NO: 44 - protein, 41 aa, 人工序列（Artificial Sequence）
  HFR3
TNYADSVKGRFTISRDDSKNTFYLQMNSLRAEDTAVYYCAR

SEQ ID NO: 45 - protein, 12 aa, 人工序列（Artificial Sequence）
  HCDR3
GSHYFGHWHFAV

SEQ ID NO: 46 - protein, 12 aa, 人工序列（Artificial Sequence）
  HCDR3
GTNYFGHWHFAV

SEQ ID NO: 47 - protein, 12 aa, 人工序列（Artificial Sequence）
  HCDR3
GTHYFGHWHFAV

SEQ ID NO: 48 - protein, 12 aa, 人工序列（Artificial Sequence）
  HCDR3
GSNYFGHWHFAV

SEQ ID NO: 49 - protein, 11 aa, 人工序列（Artificial Sequence）
  HFR4
WGQGTLVTVSS

SEQ ID NO: 50 - protein, 121 aa, 人工序列（Artificial Sequence） [sequence omitted]

SEQ ID NO: 51 - protein, 121 aa, 人工序列（Artificial Sequence）
  VH
EVQLVESGGGLVQPGGSLRLSCAVSGYSITSGYSWNWVRQAPGKGLEWVSVITYAGSTNYADSVKGRFTISRDDSKNTFYLQMNSLRAEDTAVYYCARGSHYFGHWHFAVWGQGTLVTVSS

SEQ ID NO: 52 - protein, 121 aa, 人工序列（Artificial Sequence）
  VH
EVQLVESGGGLVQPGGSLRLSCAVSGYSITSGYSWNWVRQAPGKGLEWVSVITYAGSTNYADSVKGRFTISRDDSKNTFYLQMNSLRAEDTAVYYCARGTNYFGHWHFAVWGQGTLVTVSS

SEQ ID NO: 53 - protein, 121 aa, 人工序列（Artificial Sequence）
  VH
EVQLVESGGGLVQPGGSLRLSCAVSGYSIRSGYSWNWVRQAPGKGLEWVSVITYAGSTNYADSVKGRFTISRDDSKNTFYLQMNSLRAEDTAVYYCARGSHYFGHWHFAVWGQGTLVTVSS

SEQ ID NO: 54 - protein, 121 aa, 人工序列（Artificial Sequence）
  VH
EVQLVESGGGLVQPGGSLRLSCAVSGYSITSGYSWNWVRQAPGKGLEWVSVITYAGSTNYADSVKGRFTISRDDSKNTFYLQMNSLRAEDTAVYYCARGTHYFGHWHFAVWGQGTLVTVSS

SEQ ID NO: 55 - protein, 121 aa, 人工序列（Artificial Sequence）
  VH
EVQLVESGGGLVQPGGSLRLSCAVSGYSITSGYSWNWVRQAPGKGLEWVSVITYAGSTNYADSVKGRFTISRDDSKNTFYLQMNSLRAEDTAVYYCARGSNYFGHWHFAVWGQGTLVTVSS

SEQ ID NO: 56 - protein, 121 aa, 人工序列（Artificial Sequence）
  VH
EVQLVESGGGLVQPGGSLRLSCAVSGYSITQGYSWNWVRQAPGKGLEWVSVITYAGSTNYADSVKGRFTISRDDSKNTFYLQMNSLRAEDTAVYYCARGSHYFGHWHFAVWGQGTLVTVSS

SEQ ID NO: 57 - protein, 111 aa, 人工序列（Artificial Sequence）
  VL
  misc_feature (29)..(29): Xaa = Leu或Val
  misc_feature (30)..(30): Xaa = Ala、Asp、Glu、Phe、Gly、Asn或Tyr
  misc_feature (31)..(31): Xaa = Ala、Asp、Ser或Tyr
  misc_feature (33)..(33): Xaa = Ala、Gly、Trp或Tyr
DIQLTQSPSSLSASVGDRVTITCRASQSXXXEXDSYMNWYQQKPGKAPKLLIYAASYLQSGVPSRFSGSGSGTDFTLTISSLQPEDFATYYCQQSHEDPYTFGQGTKLEIK

SEQ ID NO: 58 - protein, 121 aa, 人工序列（Artificial Sequence）
  VH
  misc_feature (30)..(30): Xaa = Arg或Thr
  misc_feature (31)..(31): Xaa = Gln或Ser
  misc_feature (100)..(100): Xaa = Ser或Thr
  misc_feature (101)..(101): Xaa = His或Asn
EVQLVESGGGLVQPGGSLRLSCAVSGYSIXXGYSWNWVRQAPGKGLEWVSVITYAGSTNYADSVKGRFTISRDDSKNTFYLQMNSLRAEDTAVYYCARGXXYFGHWHFAVWGQGTLVTVSS

SEQ ID NO: 59 - protein, 107 aa, 人工序列（Artificial Sequence） [sequence omitted]

SEQ ID NO: 60 - protein, 330 aa, 人工序列（Artificial Sequence）
  IgG1恒定区（无突变）
ASTKGPSVFPLAPSSKSTSGGTAALGCLVKDYFPEPVTVSWNSGALTSGVHTFPAVLQSSGLYSLSSVVTVPSSSLGTQTYICNVNHKPSNTKVDKKVEPKSCDKTHTCPPCPAPELLGGPSVFLFPPKPKDTLMISRTPEVTCVVVDVSHEDPEVKFNWYVDGVEVHNAKTKPREEQYNSTYRVVSVLTVLHQDWLNGKEYKCKVSNKALPAPIEKTISKAKGQPREPQVYTLPPSREEMTKNQVSLTCLVKGFYPSDIAVEWESNGQPENNYKTTPPVLDSDGSFFLYSKLTVDKSRWQQGNVFSCSVMHEALHNHYTQKSLSLSPGK

SEQ ID NO: 61 - protein, 330 aa, 人工序列（Artificial Sequence）
  IgG1恒定区（YTE突变）
ASTKGPSVFPLAPSSKSTSGGTAALGCLVKDYFPEPVTVSWNSGALTSGVHTFPAVLQSSGLYSLSSVVTVPSSSLGTQTYICNVNHKPSNTKVDKKVEPKSCDKTHTCPPCPAPELLGGPSVFLFPPKPKDTLYITREPEVTCVVVDVSHEDPEVKFNWYVDGVEVHNAKTKPREEQYNSTYRVVSVLTVLHQDWLNGKEYKCKVSNKALPAPIEKTISKAKGQPREPQVYTLPPSREEMTKNQVSLTCLVKGFYPSDIAVEWESNGQPENNYKTTPPVLDSDGSFFLYSKLTVDKSRWQQGNVFSCSVMHEALHNHYTQKSLSLSPGK

SEQ ID NO: 62 - protein, 8 aa, 人工序列（Artificial Sequence）
  HCDR1通式
  misc_feature (5)..(5): Xaa = Arg或Thr
  misc_feature (6)..(6): Xaa = Gln或Ser
GYSIXXGY

SEQ ID NO: 63 - protein, 12 aa, 人工序列（Artificial Sequence）
  HCDR3通式
  misc_feature (2)..(2): Xaa = Ser或Thr
  misc_feature (3)..(3): Xaa = His或Asn
GXXYFGHWHFAV

SEQ ID NO: 64 - protein, 15 aa, 人工序列（Artificial Sequence）
  LCDR1通式
  misc_feature (6)..(6): Xaa = Leu或Val
  misc_feature (7)..(7): Xaa = Ala、Asp、Glu、Phe、Gly、Asn或Tyr
  misc_feature (8)..(8): Xaa = Ala、Asp、Ser或Tyr
  misc_feature (10)..(10): Xaa = Ala、Gly、Trp或Tyr
RASQSXXXEXDSYMN